European Patent Specification EP 3 130 672 B1, published September 24, 2025. Title: Mutated enzyme and method for preparing terpenoid using the same. Applicant: ADEKA CORPORATION. The sequence listing filed with the application follows.

SEQUENCE LISTING (40 sequences)

SEQ ID NO: 1 - protein, 1022 aa, Saccharomycopsis fibuligera
MFSLSNYVSNWLASLARLSAHKPIHVIFLTTLLTAVAYLSVVDEYLNFDSFDISNVSFYHPPSSKDYKDWTLIEDASAYPNAARIAITPLEFRRIAKHEIPAIANTFYGVDSTEKYLISEYENAQDSIDSIRTVVSNDGTAWKIVHQYKTSKYQEYLKNAYKTLQSVIRGAETYDIAIITIAYAAMYYTFFKLFYDMRTQANSKFWLGFASASSSLFAFLLAVGTAKIFNIRVSLLSLSEGIPFLVATVGFNRIVKLSAAVLNAAAVDKESHSISLLIYRQLKDKALNFVKDQLLCAAAFVGCSIYASHLEGLRSFCLLSAFIMIYDVLLTYSYYSAVLALKVEINMIHQSIALKDALEEDGIPELAARQASLASFGSQKELSLGPNSGYVTAFKIASVAFFFAFHAYLVGSNWVFLSSNEDIIEGHNLSKSIAKHISIGSTGTVVTLLEPKIYVPKNILFQVEDLVISILEKLSTAIRDKFISKTLLFFLGTSSAINVYLLNAARAHSIDKPSQRLSKAIASKEASRRAKAAYESQKSVSKSTDDTASSEPTFDVKNILPNSGIEHTFEELVDILKNGEVSSLSNEEVTTLVVKDKLPLYALEKKLGDTTRAVAVRRQAISKLAKSPIVDSSSVPYLNYDYDKVFGACCENVIGYIPLPLGVAGPLLIDGKPFHIPMATTEGCLVASTMRGCKAINAGGGVSTVLTRDGMTRGPCVKFPSLQRAGACKIWLDSEEGQNLLKKSFNSTSRFARLQHVQTAIAGSLLFIRFRTTTGDAMGMNMISKGVEFTLKQMVEEYGWSDMDVISVSGNYCTDKKAASINWTNGRGKSIVAEARIPGEVVRKVLKSDVDALVELNVSKNLIGSAMAGSIGGFNAHAANLVTAVFLACGQDPAQNVESSNCITLIDNVDGDLQISVSMPSIEVGTIGGGTILEPQGAMLDLLGVRGPHPTTPGANAHQLAKVVASAVLAAELSLCSALAAGHLVQSHMQHNRGKPAAPAAAPSSKADVQRLTDGSKICIKS

SEQ ID NO: 2 - DNA, 3069 bp, Saccharomycopsis fibuligera
atgtttagccttagtaattatgtgtccaattggctcgcgtcattggcaaggttgtcggcacacaaaccaatccacgttatattcttaacaacgttgttaaccgctgttgcttacttgtctgtcgtcgacgagtatctcaactttgactcattcgatatctccaatgtttccttctatcatcctccatcttcaaaggactataaagattggactttaattgaggatgctagtgcttatccaaacgcagctcgtattgcaatcactccacttgagtttagaagaattgctaaacatgaaatcccggctatagcaaacactttttacggcgtcgactccaccgagaaatacttgatttctgagtacgaaaatgcccaggacagcattgactcaatcagaactgttgtttccaatgatgggactgcttggaagattgttcaccagtacaagaccagcaaatatcaagaatacctcaaaaatgcttacaaaaccttacagtctgttattcgtggtgctgaaacttatgatattgctatcattacaattgcctacgctgccatgtactacaccttttttaagctcttttatgatatgagaacccaagccaactccaagttctggttgggttttgcttcagcctcatcatctctgtttgcatttttgcttgctgttggaactgccaaaatctttaatattagagtttccttattgagcttgtctgaaggcattccatttttggttgccacggttggattcaacagaattgtaaagctttccgccgctgttttgaacgccgctgcagttgacaaagagtctcatagtatcagtttattgatttatagacaacttaaggataaagccctcaattttgtcaaagatcaattgttatgtgctgctgcatttgttgggtgctcaatttatgcatcgcacttggaaggattgagaagcttttgtttattgagtgcattcatcatgatttacgacgtgcttttgacttattcctactattctgctgtcttggctcttaaagttgaaatcaacatgattcaccaatctattgctcttaaggatgcattagaagaagacggtattcctgaacttgctgctagacaagcttctttggcatcatttgggtcacaaaaagaacttagcttgggtccaaacagcggatatgttaccgcattcaaaattgctagcgttgcatttttcttcgcattccatgcttacttagtgggcagtaactgggttttcttgagcagcaatgaggacattatcgaaggccacaacttgtccaagtcgattgctaaacatatttctattggatcaaccggtactgttgtcactttattggaaccgaaaatttacgttccaaagaacattttatttcaagttgaagatcttgttatcagtattcttgaaaaattgtctactgctatcagagataaatttattagtaagactttgcttttctttttgggtaccagttctgccatcaatgtctacttgttgaacgctgctagagcccactccattgataagccatctcaacgtcttagcaaggctattgcttcaaaagaagcatctagaagagcaaaagctgcttatgaatcacaaaagagtgtttcaaagagcaccgatgatactgctagtagcgagccaacttttgacgtaaagaatatattgccaaatagtggtattgaacatacttttgaagaattagttgacattctcaagaatggcgaagtttctagcttgtctaatgaagaagttactacccttgttgttaaagataaattgccattatatgctcttgaaaagaagttaggtgacactactcgtgctgttgctgttcgtcgtcaagctatttccaaattggccaaaagcccaattgttgatagctctagtgttccatacttgaattacgattatgataaggtgtttggcgcatgttgtgaaaacgtcattggttatattccattgcctcttggtgttgctggtccattgttaattgatggtaagccattccatattccaatggctactactgaaggttgtcttgttgcttctaccatgcgcggttgtaaagctattaatgctggtggcggtgttagcaccgtcttgactagagatggtatgacaagaggtccttgtgttaaattcccatctttgcaacgtgccggtgcttgtaagatttggttagattctgaagaaggtcaaaacttgttgaaaaaatcattcaattctacttctagatttgctagattgcaacatgttcaaactgccattgctggttctttgcttttcattagatttagaactactactggtgatgctatgggtatgaatatgatttccaaaggtgttgaatttacattgaaacaaatggttgaagaatatggttggtctgatatggatgttatctctgtttccggtaactactgtactgataagaaagccgcttctattaactggaccaatggtcgtggtaagagtattgttgctgaagctcgtattcctggagaagttgtcagaaaagttcttaagagtgacgttgatgctcttgttgaattaaacgtcagcaagaatttgattggttctgcaatggccggctctattggtggtttcaatgctcatgctgcaaatttggtcactgctgttttcttagcctgcggtcaagatcctgctcaaaatgttgaaagttccaactgtatcactttaattgataatgttgatggcgatttgcaaatatccgtttctatgccatctattgaagttggtactattggtggtggtactattcttgaacctcaaggtgctatgcttgatttattgggagttcgtggtccacatccaactactccaggggctaatgctcatcagcttgcaaaggttgttgcttctgctgttttggccgctgaattatcattgtgttcagcattggctgctggtcatttagttcaaagtcatatgcaacataaccgtggtaaacctgctgctccagcggccgctccatcaagcaaggctgatgttcagcgtttgactgatggatcaaagatctgtatcaaatcttaa

SEQ ID NO: 3 - DNA, 41 bp, Artificial Sequence
  FL HMGR primer-1
aatcaactggtacccgggatgtttagccttagtaattatgt

SEQ ID NO: 4 - DNA, 44 bp, Artificial Sequence
  FL HMGR primer-2
ttagttaacctctagagctcttaagatttgatacagatctttga

SEQ ID NO: 5 - DNA, 19 bp, Artificial Sequence
  HGMR seq primer-1
tctgcacaatatttcaagc

SEQ ID NO: 6 - DNA, 24 bp, Artificial Sequence
  HGMR seq primer-2
ttcgttttaaaacctaagagtcac

SEQ ID NO: 7 - DNA, 45 bp, Artificial Sequence
  tHGMR primer-1
aatcaactggtacccgggatgtctcaacgtcttagcaaggctatt

SEQ ID NO: 8 - DNA, 44 bp, Artificial Sequence; identical to SEQ ID NO: 4
  tHGMR primer-1

SEQ ID NO: 9 - DNA, 39 bp, Artificial Sequence
  tHGMR primer-3
aatcaactggtacccgggatggaccaattggtgaaaact

SEQ ID NO: 10 - DNA, 35 bp, Artificial Sequence
  tHGMR primer-4
ttagttaacctctagagctcttaggatttaatgca

SEQ ID NO: 11 - DNA, 33 bp, Artificial Sequence
  S820A primer-1
gccattaactggaccaatggtcgtggtaagagt

SEQ ID NO: 12 - DNA, 33 bp, Artificial Sequence
  S820A primer-2
ggtccagttaatggcagcggctttcttatcagt

SEQ ID NO: 13 - DNA, 33 bp, Artificial Sequence
  T824I primer-1
tctattaactggatcaatggtcgtggtaagagt

SEQ ID NO: 14 - DNA, 33 bp, Artificial Sequence
  T824I primer-2
gatccagttaatagaagcggctttcttatcagt

SEQ ID NO: 15 - DNA, 33 bp, Artificial Sequence
  S820A/T824I primer-1
gccattaactggatcaatggtcgtggtaagagt

SEQ ID NO: 16 - DNA, 33 bp, Artificial Sequence
  S820A/T824I primer-2
gatccagttaatggcagcggctttcttatcagt

SEQ ID NO: 17 - DNA, 27 bp, Artificial Sequence
  S744A primer-1
tgaaaaaagctttcaattctacttcta

SEQ ID NO: 18 - DNA, 27 bp, Artificial Sequence
  S744A primer-2
attgaaagcttttttcaacaagttttg

SEQ ID NO: 19 - DNA, 27 bp, Artificial Sequence
  A818P primer-1
tgataagaaaccagcttctattaactg

SEQ ID NO: 20 - DNA, 27 bp, Artificial Sequence
  A818P primer-2
gctggtttcttatcagtacagtagtta

SEQ ID NO: 21 - DNA, 28 bp, Artificial Sequence
  N825E primer-1
tggaccgaaggtcgtggtaagagtattg

SEQ ID NO: 22 - DNA, 28 bp, Artificial Sequence
  N825E primer-2
acgaccttcggtccagttaatagaagcg

SEQ ID NO: 23 - DNA, 33 bp, Artificial Sequence
  A852S-I856T primer-1
tctatcaactggaccgaaggtcgtggtaagagt

SEQ ID NO: 24 - DNA, 33 bp, Artificial Sequence
  A852S-I856T primer-2
ggtccagttgatagaagctggttttttgtcggt

SEQ ID NO: 25 - DNA, 27 bp, Artificial Sequence
  A776S primer-1
aaaaaatcatttaactctacatcaaga

SEQ ID NO: 26 - DNA, 28 bp, Artificial Sequence
  A776S primer-2
gttaaatgattttttaatttgcgttttg

SEQ ID NO: 27 - DNA, 27 bp, Artificial Sequence
  E857N primer-1
tggaccaatggtcgtggtaagagtgtc

SEQ ID NO: 28 - DNA, 27 bp, Artificial Sequence
  E857N primer-2
acgaccattggtccagttgatagaagc

SEQ ID NO: 29 - DNA, 27 bp, Artificial Sequence
  P850A primer-1
cgacaaaaaagccgcttctatcaactg

SEQ ID NO: 30 - DNA, 27 bp, Artificial Sequence
  P850A primer-2
gcggcttttttgtcggtacagtagtta

SEQ ID NO: 31 - DNA, 28 bp, Artificial Sequence
  A772L-I773L primer-1
aaaacttgttgaaaaaatcatttaactc

SEQ ID NO: 32 - DNA, 27 bp, Artificial Sequence
  A772L-I773L primer-2
ttttcaacaagttttgtccctcttctg

SEQ ID NO: 33 - DNA, 28 bp, Artificial Sequence
  L740A primer-1
aaaacgcattgaaaaaatcattcaattc

SEQ ID NO: 34 - DNA, 29 bp, Artificial Sequence
  L740A primer-2
ttttcaatgcgttttgaccttcttcagta

SEQ ID NO: 35 - DNA, 27 bp, Artificial Sequence
  L741I primer-1
acttgattaaaaaatcattcaattcta

SEQ ID NO: 36 - DNA, 29 bp, Artificial Sequence
  L741I primer-2
attttttaatcaagttttgaccttcttca

SEQ ID NO: 37 - DNA, 27 bp, Artificial Sequence
  L773L primer-1
acgcattgaaaaaatcatttaactcta

SEQ ID NO: 38 - DNA, 28 bp, Artificial Sequence
  L773L primer-2
attttttcaatgcgttttgtccctcttc

SEQ ID NO: 39 - DNA, 27 bp, Artificial Sequence
  T856I primer-1
aactggatcaatggtcgtggtaagagt

SEQ ID NO: 40 - DNA, 27 bp, Artificial Sequence
  T856I primer-2
accattgatccagttgatagaagcggc